European Patent Specification EP 3 827 016 B1, published December 3, 2025. Title: Antibodies to Granulocyte-Macrophage Colony Stimulating Factor and Uses Thereof. Applicant: ELIXIRON IMMUNOTHERAPEUTICS (HONG KONG) LIMITED. The sequence listing filed with the application follows.

SEQUENCE LISTING (15 sequences)

SEQ ID NO: 1 - protein, 121 aa, Artificial Sequence
  Heavy chain variable domain sequence of 1D2
QVQLVQSGAEVKKPGASVKVSCEASGYTFTDKYLHWVRQAPGQGLEWMAWINPKSGGTFYAQNFKGRVTVTRDTSINTAYLELTSLRLDDTSTYYCARGRDYYDQGAADLWGQGTMVTVSS

SEQ ID NO: 2 - protein, 108 aa, Artificial Sequence
  Light chain variable domain sequence of 1D2
DIQLTQSPSSLSASVGDRVTITCRASQGINSVLAWYQQKPGKAPKLLLYAASKLESGVPSRFSGSGSGTDYTLTISSLQPEDFGTYYCQQYYSPVRTFGQGTKVEIKR

SEQ ID NO: 3 - protein, 121 aa, Artificial Sequence
  Heavy chain variable domain sequences with D89E (ED) mutation
QVQLVQSGAEVKKPGASVKVSCEASGYTFTDKYLHWVRQAPGQGLEWMAWINPKSGGTFYAQNFKGRVTVTRDTSINTAYLELTSLRLEDTSTYYCARGRDYYDQGAADLWGQGTMVTVSS

SEQ ID NO: 4 - protein, 121 aa, Artificial Sequence
  Heavy chain variable domain sequences with D90E (DE) mutation
QVQLVQSGAEVKKPGASVKVSCEASGYTFTDKYLHWVRQAPGQGLEWMAWINPKSGGTFYAQNFKGRVTVTRDTSINTAYLELTSLRLDETSTYYCARGRDYYDQGAADLWGQGTMVTVSS

SEQ ID NO: 5 - protein, 8 aa, Artificial Sequence
  Heavy chain CDR1 of 1D2
GYTFTDKY

SEQ ID NO: 6 - protein, 8 aa, Artificial Sequence
  Heavy chain CDR2 of 1D2
INPKSGGT

SEQ ID NO: 7 - protein, 14 aa, Artificial Sequence
  Heavy chain CDR3 of 1D2
ARGRDYYDQGAADL

SEQ ID NO: 8 - protein, 6 aa, Artificial Sequence
  Light chain CDR1 of 1D2
QGINSV

SEQ ID NO: 9 - protein, 3 aa, Artificial Sequence
  Light chain CDR2 of 1D2
AAS

SEQ ID NO: 10 - protein, 9 aa, Artificial Sequence
  Light chain CDR3 of 1D2
QQYYSPVRT

SEQ ID NO: 11 - protein, 8 aa, Artificial Sequence
  Variations in HC CDR1
  MUTAGEN (6)..(6): X can be D, E, S, P, G, A, V, N, Q, C, W, R, T, or L
  MUTAGEN (7)..(7): X can be K, V, L, E, P, S, T, C, D, R, H, A, F, Q, or N
GYTFTXXY

SEQ ID NO: 12 - protein, 8 aa, Artificial Sequence
  Variations in in HC CDR2
  MUTAGEN (4)..(4): X can be K, L, M, E, H, S, V, N, C, F, P, W, G, A, I, R, T or Q
INPXSGGT

SEQ ID NO: 13 - protein, 14 aa, Artificial Sequence
  Variations in HC CDR3
  MUTAGEN (4)..(4): X can be R, V, S, A, C, L, P, I, T, G, M, E, or Q
  MUTAGEN (6)..(6): X can be: Y, I, L, W, F, T, V, A, G, N, Y, or S
  MUTAGEN (7)..(7): X can be Y, N, P, S, K, R, G, W, D, Q, L, H, F, A, T, V, or M
  MUTAGEN (9)..(9): X can be Q, S, T, M, N, G, V, L, E, or W
ARGXDXXDXGAADL

SEQ ID NO: 14 - protein, 6 aa, Artificial Sequence
  Variations in LC CDR1
  MUTAGEN (6)..(6): X can be V, L, G, E, R, F, P, H, or Y
QGINSX

SEQ ID NO: 15 - protein, 9 aa, Artificial Sequence
  Variations in LC CDR 3
  MUTAGEN (6)..(6): X can be P, R, N, or C
  MUTAGEN (7)..(7): X can be V, C, D. L, E, P, or R
QQYYSXXRT